European Patent Specification EP 4 313 114 B1, published September 17, 2025. Title: Combined treatment of brain injury. Applicant: Chiesi Farmaceutici S.p.A. The sequence listing filed with the application follows.

SEQUENCE LISTING (5 sequences)

SEQ ID NO: 1 - protein, 118 aa, Artificial Sequence
  synthetic
SSSHPIFHRGEFSVCDSVSVWVGDKTTATDIKGKEVMVLGEVNINNSVFKQYFFETKCRDSNPVDSGCRGIDSKHWNSYCTTTHTFVKALTMDGKQAAWEFIRIDTACVCVLSRKAVR

SEQ ID NO: 2 - protein, 9 aa, Artificial Sequence
  synthetic
SSSHPIFHR

SEQ ID NO: 3 - protein, 8 aa, Artificial Sequence
  synthetic
QAAWEFIR

SEQ ID NO: 4 - protein, 7 aa, Artificial Sequence
  synthetic
QYFFETK

SEQ ID NO: 5 - protein, 7 aa, Artificial Sequence
  synthetic
ALTTDDK